European Patent Specification EP 3 601 604 B1, published February 19, 2025. Title: MULTIPLEX ISOTYPE-SPECIFIC ANTIBODY DETECTION. Applicant: The Board of Trustees of the Leland Stanford Junior University. The sequence listing filed with the application follows.

SEQUENCE LISTING (21 sequences)

SEQ ID NO: 1 - DNA, 40 bp, Artificial Sequence
  DNA 1A
  source (1)..(40): sequence is synthesized
caggtagtagtacgtctgtttcacgatgagactggatgaa

SEQ ID NO: 2 - DNA, 40 bp, Artificial Sequence
  DNA 1B
  source (1)..(40): sequence is synthesized
tcacggtagcataaggtgcaagataatactctcgcagcac

SEQ ID NO: 3 - DNA, 20 bp, Artificial Sequence
  Reverse primer 1
  source (1)..(20): sequence is synthesized
gtgctgcgagagtattatct

SEQ ID NO: 4 - DNA, 20 bp, Artificial Sequence
  Forward primer 1
  source (1)..(20): sequence is synthesized
caggtagtagtacgtctgtt

SEQ ID NO: 5 - DNA, 40 bp, Artificial Sequence
  DNA 2A
  source (1)..(40): sequence is synthesized
ggcctcctccaattaaagaatcacgatgagactggatgaa

SEQ ID NO: 6 - DNA, 40 bp, Artificial Sequence
  DNA 2B
  source (1)..(40): sequence is synthesized
tcacggtagcataaggtgcagtacccaaataacggttcac

SEQ ID NO: 7 - DNA, 20 bp, Artificial Sequence
  Reverse primer 2
  source (1)..(20): sequence is synthesized
gtgaaccgttatttgggtac

SEQ ID NO: 8 - DNA, 20 bp, Artificial Sequence
  Forward primer 2
  source (1)..(20): sequence is synthesized
ggcctcctccaattaaagaa

SEQ ID NO: 9 - DNA, 40 bp, Artificial Sequence
  DNA 3A
  source (1)..(40): sequence is synthesized
ggatcactccaactagactatcacgatgagactggatgaa

SEQ ID NO: 10 - DNA, 40 bp, Artificial Sequence
  DNA 3B
  source (1)..(40): sequence is synthesized
tcacggtagcataaggtgcagttatatctgccactgtcac

SEQ ID NO: 11 - DNA, 20 bp, Artificial Sequence
  Reverse primer 3
  source (1)..(20): sequence is synthesized
gtgacagtggcagatataac

SEQ ID NO: 12 - DNA, 20 bp, Artificial Sequence
  Forward primer 3
  source (1)..(20): sequence is synthesized
ggatcactccaactagacta

SEQ ID NO: 13 - DNA, 40 bp, Artificial Sequence
  DNA 4A
  source (1)..(40): sequence is synthesized
agagtccacttcccataatgtcacgatgagactggatgaa

SEQ ID NO: 14 - DNA, 40 bp, Artificial Sequence
  DNA 4B
  source (1)..(40): sequence is synthesized
tcacggtagcataaggtgcacggtactgtcagcatagttc

SEQ ID NO: 15 - DNA, 20 bp, Artificial Sequence
  Reverse primer 4
  source (1)..(20): sequence is synthesized
gaactatgctgacagtaccg

SEQ ID NO: 16 - DNA, 20 bp, Artificial Sequence
  Forward primer 4
  source (1)..(20): sequence is synthesized
agagtccacttcccataatg

SEQ ID NO: 17 - DNA, 40 bp, Artificial Sequence
  DNA 5A
  source (1)..(40): sequence is synthesized
ctacgactaggagatagatgtcacgatgagactggatgaa

SEQ ID NO: 18 - DNA, 40 bp, Artificial Sequence
  DNA 5B
  source (1)..(40): sequence is synthesized
tcacggtagcataaggtgcagttatgtatagtacgctcgc

SEQ ID NO: 19 - DNA, 20 bp, Artificial Sequence
  Reverse primer 5
  source (1)..(20): sequence is synthesized
gcgagcgtactatacataac

SEQ ID NO: 20 - DNA, 20 bp, Artificial Sequence
  Forward primer 5
  source (1)..(20): sequence is synthesized
ctacgactaggagatagatg

SEQ ID NO: 21 - DNA, 18 bp, Artificial Sequence
  Bridge oligo
  source (1)..(18): sequence is synthesized
ctaccgtgattcatccag